European Patent Application EP 4 516 311 A1, published March 5, 2025. Title: SEQUÊNCIA DE ÁCIDO NUCLEICO QUE CODIFICA UM RECEPTOR DE CÉLULA NATURAL KILLER DE ANTÍGENO QUIMÉRICO (NK-CAR), POLIPEPTÍDEO DO REFERIDO NK CAR, VETOR QUE COMPREENDE A REFERIDA SEQUÊNCIA DE ÁCIDO NUCLEICO, MÉTODO IN VITRO DE OBTENÇÃO DE UMA CÉLULA NK, USO DOS REFERIDOS SEQUÊNCIA DE ÁCIDO NUCLEICA, POLIPEPTÍDEO OU VETOR, E COMPOSIÇÃO FARMACÊUTICA. Applicant: FUNDAÇÃO HEMOCENTRO DE RIBEIRÃO PRETO. The sequence listing filed with the application follows.

SEQUENCE LISTING (20 sequences)

SEQ ID NO: 1 - protein, 271 aa, Murine
MYRMQLLSCIALSLALVTNSDIQLTQSPASLAVSLGQRATISCKASQSVDYDGDSYLNWYQQIPGQPPKLLIYDASNLVSGIPPRFSGSGSGTDFTLNIHPVEKVDAATYHCQQSTEDPWTFGGGTKLEIKGGGGSGGGGSGGGGSQVQLQQSGAELVRPGSSVKISCKASGYAFSSYWMNWVKQRPGQGLEWIGQIWPGDGDTNYNGKFKGKATLTADESSSTAYMQLSSLASEDSAVYFCARRETTTVGRYYYAMDYWGQGTTVTVSSS

SEQ ID NO: 2 - DNA, 813 bp, Murine
  source 1..813: mol_type = other DNA
atgtacaggatgcaactcctgtcttgcattgcactaagtcttgcacttgtcacgaattccgatatccagctgacccagtctccagcttctttggctgtgtctctagggcagagggccaccatctcctgcaaggccagccaaagtgttgattatgatggtgatagttatttgaactggtaccagcagatcccaggacagccccctaagctgctgatctacgacgctagtaatctggtgtcaggaatcccacccaggttcagcggttctggcagtggaactgattttaccctgaacattcaccccgtggagaaagtcgacgccgctacctatcattgccagcagtccacagaggacccctggactttcggcggagggaccaaactggaaatcaagggtggcggagggtctggtggcggagggagtggtggcggagggtcccaggtgcagctgcagcagtccggagctgaactggtgagacccggctccagcgtcaaaatttcctgtaaggctagcggatatgcattttctagttactggatgaattgggtgaagcagcgacctggacagggtctggagtggatcggccagatttggccaggcgatggagacaccaactacaatgggaagttcaaaggcaaggccaccctgacagctgacgaatcatccagcacagcatatatgcagctgtctagtctggcaagcgaggattctgccgtgtacttttgtgctaggcgggaaaccacaactgtcggcagatactattacgctatggactactgggggcagggaacaactgtgaccgtgagcagctcg

SEQ ID NO: 3 - protein, 69 aa, Homo sapiens
TTTPAPRPPTPAPTIASQPLSLRPEACRPAAGGAVHTRGLDFACDIYIWAPLAGTCGVLLLSLVITLYC

SEQ ID NO: 4 - DNA, 207 bp, Homo sapiens
  source 1..207: mol_type = other DNA
accacgacgccagcgccgcgaccaccaacaccggcgcccaccatcgcgtcgcagcccctgtccctgcgcccagaggcgtgccggccagcggcggggggcgcagtgcacacgagggggctggacttcgcctgtgatatctacatctgggcgcccttggccgggacttgtggggtccttctcctgtcactggttatcaccctttactgc

SEQ ID NO: 5 - protein, 42 aa, Homo sapiens
KRGRKKLLYIFKQPFMRPVQTTQEEDGCSCRFPEEEEGGCEL

SEQ ID NO: 6 - DNA, 126 bp, Homo sapiens
  source 1..126: mol_type = other DNA
aaacggggcagaaagaaactcctgtatatattcaaacaaccatttatgagaccagtacaaactactcaagaggaagatggctgtagctgccgatttccagaagaagaagaaggaggatgtgaactg

SEQ ID NO: 7 - protein, 112 aa, Homo sapiens
RVKFSRSADAPAYKQGQNQLYNELNLGRREEYDVLDKRRGRDPEMGGKPRRKNPQEGLYNELQKDKMAEAYSEIGMKGERRRGKGHDGLYQGLSTATKDTYDALHMQALPPR

SEQ ID NO: 8 - DNA, 336 bp, Homo sapiens
  source 1..336: mol_type = other DNA
agagtgaagttcagcaggagcgcagacgcccccgcgtacaagcagggccagaaccagctctataacgagctcaatctaggacgaagagaggagtacgatgttttggacaagaggcgtggccgggaccctgagatggggggaaagccgagaaggaagaaccctcaggaaggcctgtacaatgaactgcagaaagataagatggcggaggcctacagtgagattgggatgaaaggcgagcgccggaggggcaaggggcacgatggcctttaccagggtctcagtacagccaccaaggacacctacgacgcccttcacatgcaggccctgccccctcgc

SEQ ID NO: 9 - protein, 18 aa, synthetic construct
  REGION 1..18: note = peptdeo de autoclivagem
EGRGSLLTCGDVEENPGP

SEQ ID NO: 10 - DNA, 54 bp, synthetic construct
  misc_feature 1..54: note = peptdeo de autoclivagem
  source 1..54: mol_type = other DNA
gagggcaggggaagtcttctaacatgcggggacgtggaggaaaatcccggccca

SEQ ID NO: 11 - DNA, 1197 bp, synthetic construct
  misc_feature 1..1197: note = interleucina-15 com seu receptor RA
  source 1..1197: mol_type = other DNA
atggtattgggaaccatagatttgtgcagctgtttcagtgcagggcttcctaaaacagaagccaactgggtgaatgtaataagtgatttgaaaaaaattgaagatcttattcaatctatgcatattgatgctactttatatacggaaagtgatgttcaccccagttgcaaagtaacagcaatgaagtgctttctcttggagttacaagttatttcacttgagtccggagatgcaagtattcatgatacagtagaaaatctgatcatcctagcaaacaacagtttgtcttctaatgggaatgtaacagaatctggatgcaaagaatgtgaggaactggaggaaaaaaatattaaagaatttttgcagagttttgtacatattgtccaaatgttcatcaacacttctagcggcggcggcagcggcggcggcggcagcggcggcggcggcagcggcggcggcggcagcggcggcggcagcctgcagatcacgtgccctccccccatgtccgtggaacacgcagacatctgggtcaagagctacagcttgtactccagggagcggtacatttgtaactctggtttcaagcgtaaagccggcacgtccagcctgacggagtgcgtgttgaacaaggccacgaatgtcgcccactggacaacccccagtctcaaatgcattagagaccctgccctggttcaccaaaggccagcgccaccctccacagtaacgacggcaggggtgaccccacagccagagagcctctccccttctggaaaagagcccgcagcttcatctcccagctcaaacaacacagcggccacaacagcagctattgtcccgggctcccagctgatgccttcaaaatcaccttccacaggaaccacagagataagcagtcatgagtcctcccacggcaccccctctcagacaacagccaagaactgggaactcacagcatccgcctcccaccagccgccaggtgtgtatccacagggccacagcgacaccactgtggctatctccacgtccactgtcctgctgtgtgggctgagcgctgtgtctctcctggcatgctacctcaagtcaaggcaaactcccccgctggccagcgttgaaatggaagccatggaggctctgccggtgacttgggggaccagcagcagagatgaagacttggaaaactgctctcaccacctatga

SEQ ID NO: 12 - DNA, 1362 bp, synthetic construct
  misc_feature 1..1362: note = IL-27 com ligante de elastina
  source 1..1362: mol_type = other DNA
atgaccccgcagcttctcctggcccttgtcctctgggccagctgcccgccctgcagtggaaggaaagggcccccagcagctctgacactgccccgggtgcaatgccgagcctctcggtacccgatcgccgtggattgctcctggaccctgccgcctgctccaaactccaccagccccgtgtccttcattgccacgtacaggctcggcatggctgcccggggccacagctggccctgcctgcagcagacgccaacgtccaccagctgcaccatcacggatgtccagctgttctccatggctccctacgtgctcaatgtcaccgccgtccacccctggggctccagcagcagcttcgtgcctttcataacagagcacatcatcaagcccgaccctccagaaggcgtgcgcctaagccccctcgctgagcgccagctacaggtgcagtgggagcctcccgggtcctggcccttcccagagatcttctcactgaagtactggatccgttacaagcgtcagggagctgcgcgcttccaccgggtggggcccattgaagccacgtccttcatcctcagggctgtgcggccccgagccaggtactacatccaagtggcggctcaggacctcacagactacggggaactgagtgactggagtctccccgccactgccacaatgagcctgggcaaggttcctggagtaggggtacctggagtgggcttcccaaggcccccagggaggccccagctgagcctgcaggagctgcggagggagttcacagtcagcctgcatctcgccaggaagctgctcgccgaggttcggggccaggcccaccgctttgcggaatctcacctgccaggagtgaacctgtacctcctgcccctgggagagcagctccctgatgtttccctgaccttccaggcctggcgccgcctctctgacccggagcgtctctgcttcatctccaccacgcttcagcccttccatgccctgctgggagggctggggacccagggccgctggaccaacatggagaggatgcagctgtgggccatgaggctggacctccgcgatctgcagcggcacctccgcttccaggtgctggctgcaggattcaacctcccggaggaggaggaggaggaagaggaggaggaggaggaggagaggaaggggctgctcccaggggcactgggcagcgccttacagggcccggcccaggtgtcctggccccagctcctctccacctaccgcctgctgcactccttggagctcgtcttatctcgggccgtgcgggagttgctgctgctgtccaaggctgggcactcagtctggcccttggggttcccaacattgagcccccagccc

SEQ ID NO: 13 - protein, 398 aa, synthetic construct
  REGION 1..398: note = interleucina-15 com seu receptor RA (IL-15RA)
MVLGTIDLCSCFSAGLPKTEANWVNVISDLKKIEDLIQSMHIDATLYTESDVHPSCKVTAMKCFLLELQVISLESGDASIHDTVENLIILANNSLSSNGNVTESGCKECEELEEKNIKEFLQSFVHIVQMFINTSSGGGSGGGGSGGGGSGGGGSGGGSLQITCPPPMSVEHADIWVKSYSLYSRERYICNSGFKRKAGTSSLTECVLNKATNVAHWTTPSLKCIRDPALVHQRPAPPSTVTTAGVTPQPESLSPSGKEPAASSPSSNNTAATTAAIVPGSQLMPSKSPSTGTTEISSHESSHGTPSQTTAKNWELTASASHQPPGVYPQGHSDTTVAISTSTVLLCGLSAVSLLACYLKSRQTPPLASVEMEAMEALPVTWGTSSRDEDLENCSHHL

SEQ ID NO: 14 - protein, 454 aa, synthetic construct
  REGION 1..454: note = interleucina-27 (IL-27)
MTPQLLLALVLWASCPPCSGRKGPPAALTLPRVQCRASRYPIAVDCSWTLPPAPNSTSPVSFIATYRLGMAARGHSWPCLQQTPTSTSCTITDVQLFSMAPYVLNVTAVHPWGSSSSFVPFITEHIIKPDPPEGVRLSPLAERQLQVQWEPPGSWPFPEIFSLKYWIRYKRQGAARFHRVGPIEATSFILRAVRPRARYYIQVAAQDLTDYGELSDWSLPATATMSLGKVPGVGVPGVGFPRPPGRPQLSLQELRREFTVSLHLARKLLAEVRGQAHRFAESHLPGVNLYLLPLGEQLPDVSLTFQAWRRLSDPERLCFISTTLQPFHALLGGLGTQGRWTNMERMQLWAMRLDLRDLQRHLRFQVLAAGFNLPEEEEEEEEEEEEERKGLLPGALGSALQGPAQVSWPQLLSTYRLLHSLELVLSRAVRELLLLSKAGHSVWPLGFPTLSPQP

SEQ ID NO: 15 - DNA, 2745 bp, synthetic construct
  misc_feature 1..2745: note = CAR Cd19/IL15RA
  source 1..2745: mol_type = other DNA
atgtacaggatgcaactcctgtcttgcattgcactaagtcttgcacttgtcacgaattccgatatccagctgacccagtctccagcttctttggctgtgtctctagggcagagggccaccatctcctgcaaggccagccaaagtgttgattatgatggtgatagttatttgaactggtaccagcagatcccaggacagccccctaagctgctgatctacgacgctagtaatctggtgtcaggaatcccacccaggttcagcggttctggcagtggaactgattttaccctgaacattcaccccgtggagaaagtcgacgccgctacctatcattgccagcagtccacagaggacccctggactttcggcggagggaccaaactggaaatcaagggtggcggagggtctggtggcggagggagtggtggcggagggtcccaggtgcagctgcagcagtccggagctgaactggtgagacccggctccagcgtcaaaatttcctgtaaggctagcggatatgcattttctagttactggatgaattgggtgaagcagcgacctggacagggtctggagtggatcggccagatttggccaggcgatggagacaccaactacaatgggaagttcaaaggcaaggccaccctgacagctgacgaatcatccagcacagcatatatgcagctgtctagtctggcaagcgaggattctgccgtgtacttttgtgctaggcgggaaaccacaactgtcggcagatactattacgctatggactactgggggcagggaacaactgtgaccgtgagcagctcgaccacgacgccagcgccgcgaccaccaacaccggcgcccaccatcgcgtcgcagcccctgtccctgcgcccagaggcgtgccggccagcggcggggggcgcagtgcacacgagggggctggacttcgcctgtgatatctacatctgggcgcccttggccgggacttgtggggtccttctcctgtcactggttatcaccctttactgcaaacggggcagaaagaaactcctgtatatattcaaacaaccatttatgagaccagtacaaactactcaagaggaagatggctgtagctgccgatttccagaagaagaagaaggaggatgtgaactgagagtgaagttcagcaggagcgcagacgcccccgcgtacaagcagggccagaaccagctctataacgagctcaatctaggacgaagagaggagtacgatgttttggacaagaggcgtggccgggaccctgagatggggggaaagccgagaaggaagaaccctcaggaaggcctgtacaatgaactgcagaaagataagatggcggaggcctacagtgagattgggatgaaaggcgagcgccggaggggcaaggggcacgatggcctttaccagggtctcagtacagccaccaaggacacctacgacgcccttcacatgcaggccctgccccctcgcttaggctccggcgagggcaggggaagtcttctaacatgcggggacgtggaggaaaatcccggcccaatggtattgggaaccatagatttgtgcagctgtttcagtgcagggcttcctaaaacagaagccaactgggtgaatgtaataagtgatttgaaaaaaattgaagatcttattcaatctatgcatattgatgctactttatatacggaaagtgatgttcaccccagttgcaaagtaacagcaatgaagtgctttctcttggagttacaagttatttcacttgagtccggagatgcaagtattcatgatacagtagaaaatctgatcatcctagcaaacaacagtttgtcttctaatgggaatgtaacagaatctggatgcaaagaatgtgaggaactggaggaaaaaaatattaaagaatttttgcagagttttgtacatattgtccaaatgttcatcaacacttctagcggcggcggcagcggcggcggcggcagcggcggcggcggcagcggcggcggcggcagcggcggcggcagcctgcagatcacgtgccctccccccatgtccgtggaacacgcagacatctgggtcaagagctacagcttgtactccagggagcggtacatttgtaactctggtttcaagcgtaaagccggcacgtccagcctgacggagtgcgtgttgaacaaggccacgaatgtcgcccactggacaacccccagtctcaaatgcattagagaccctgccctggttcaccaaaggccagcgccaccctccacagtaacgacggcaggggtgaccccacagccagagagcctctccccttctggaaaagagcccgcagcttcatctcccagctcaaacaacacagcggccacaacagcagctattgtcccgggctcccagctgatgccttcaaaatcaccttccacaggaaccacagagataagcagtcatgagtcctcccacggcaccccctctcagacaacagccaagaactgggaactcacagcatccgcctcccaccagccgccaggtgtgtatccacagggccacagcgacaccactgtggctatctccacgtccactgtcctgctgtgtgggctgagcgctgtgtctctcctggcatgctacctcaagtcaaggcaaactcccccgctggccagcgttgaaatggaagccatggaggctctgccggtgacttgggggaccagcagcagagatgaagacttggaaaactgctctcaccacctatga

SEQ ID NO: 16 - DNA, 2916 bp, synthetic construct
  misc_feature 1..2916: note = CAR Cd19/IL27
  source 1..2916: mol_type = other DNA
atgtacaggatgcaactcctgtcttgcattgcactaagtcttgcacttgtcacgaattccgatatccagctgacccagtctccagcttctttggctgtgtctctagggcagagggccaccatctcctgcaaggccagccaaagtgttgattatgatggtgatagttatttgaactggtaccagcagatcccaggacagccccctaagctgctgatctacgacgctagtaatctggtgtcaggaatcccacccaggttcagcggttctggcagtggaactgattttaccctgaacattcaccccgtggagaaagtcgacgccgctacctatcattgccagcagtccacagaggacccctggactttcggcggagggaccaaactggaaatcaagggtggcggagggtctggtggcggagggagtggtggcggagggtcccaggtgcagctgcagcagtccggagctgaactggtgagacccggctccagcgtcaaaatttcctgtaaggctagcggatatgcattttctagttactggatgaattgggtgaagcagcgacctggacagggtctggagtggatcggccagatttggccaggcgatggagacaccaactacaatgggaagttcaaaggcaaggccaccctgacagctgacgaatcatccagcacagcatatatgcagctgtctagtctggcaagcgaggattctgccgtgtacttttgtgctaggcgggaaaccacaactgtcggcagatactattacgctatggactactgggggcagggaacaactgtgaccgtgagcagctcgaccacgacgccagcgccgcgaccaccaacaccggcgcccaccatcgcgtcgcagcccctgtccctgcgcccagaggcgtgccggccagcggcggggggcgcagtgcacacgagggggctggacttcgcctgtgatatctacatctgggcgcccttggccgggacttgtggggtccttctcctgtcactggttatcaccctttactgcaaacggggcagaaagaaactcctgtatatattcaaacaaccatttatgagaccagtacaaactactcaagaggaagatggctgtagctgccgatttccagaagaagaagaaggaggatgtgaactgagagtgaagttcagcaggagcgcagacgcccccgcgtacaagcagggccagaaccagctctataacgagctcaatctaggacgaagagaggagtacgatgttttggacaagaggcgtggccgggaccctgagatggggggaaagccgagaaggaagaaccctcaggaaggcctgtacaatgaactgcagaaagataagatggcggaggcctacagtgagattgggatgaaaggcgagcgccggaggggcaaggggcacgatggcctttaccagggtctcagtacagccaccaaggacacctacgacgcccttcacatgcaggccctgccccctcgcttaggctccggcgagggcaggggaagtcttctaacatgcggggacgtggaggaaaatcccggcccaatgaccccgcagcttctcctggcccttgtcctctgggccagctgcccgccctgcagtggaaggaaagggcccccagcagctctgacactgccccgggtgcaatgccgagcctctcggtacccgatcgccgtggattgctcctggaccctgccgcctgctccaaactccaccagccccgtgtccttcattgccacgtacaggctcggcatggctgcccggggccacagctggccctgcctgcagcagacgccaacgtccaccagctgcaccatcacggatgtccagctgttctccatggctccctacgtgctcaatgtcaccgccgtccacccctggggctccagcagcagcttcgtgcctttcataacagagcacatcatcaagcccgaccctccagaaggcgtgcgcctaagccccctcgctgagcgccagctacaggtgcagtgggagcctcccgggtcctggcccttcccagagatcttctcactgaagtactggatccgttacaagcgtcagggagctgcgcgcttccaccgggtggggcccattgaagccacgtccttcatcctcagggctgtgcggccccgagccaggtactacatccaagtggcggctcaggacctcacagactacggggaactgagtgactggagtctccccgccactgccacaatgagcctgggcaaggttcctggagtaggggtacctggagtgggcttcccaaggcccccagggaggccccagctgagcctgcaggagctgcggagggagttcacagtcagcctgcatctcgccaggaagctgctcgccgaggttcggggccaggcccaccgctttgcggaatctcacctgccaggagtgaacctgtacctcctgcccctgggagagcagctccctgatgtttccctgaccttccaggcctggcgccgcctctctgacccggagcgtctctgcttcatctccaccacgcttcagcccttccatgccctgctgggagggctggggacccagggccgctggaccaacatggagaggatgcagctgtgggccatgaggctggacctccgcgatctgcagcggcacctccgcttccaggtgctggctgcaggattcaacctcccggaggaggaggaggaggaagaggaggaggaggaggaggagaggaaggggctgctcccaggggcactgggcagcgccttacagggcccggcccaggtgtcctggccccagctcctctccacctaccgcctgctgcactccttggagctcgtcttatctcgggccgtgcgggagttgctgctgctgtccaaggctgggcactcagtctggcccttggggttcccaacattgagcccccagcccaactag

SEQ ID NO: 17 - protein, 914 aa, synthetic construct
  REGION 1..914: note = CAR Cd19/IL15RA
MYRMQLLSCIALSLALVTNSDIQLTQSPASLAVSLGQRATISCKASQSVDYDGDSYLNWYQQIPGQPPKLLIYDASNLVSGIPPRFSGSGSGTDFTLNIHPVEKVDAATYHCQQSTEDPWTFGGGTKLEIKGGGGSGGGGSGGGGSQVQLQQSGAELVRPGSSVKISCKASGYAFSSYWMNWVKQRPGQGLEWIGQIWPGDGDTNYNGKFKGKATLTADESSSTAYMQLSSLASEDSAVYFCARRETTTVGRYYYAMDYWGQGTTVTVSSSTTTPAPRPPTPAPTIASQPLSLRPEACRPAAGGAVHTRGLDFACDIYIWAPLAGTCGVLLLSLVITLYCKRGRKKLLYIFKQPFMRPVQTTQEEDGCSCRFPEEEEGGCELRVKFSRSADAPAYKQGQNQLYNELNLGRREEYDVLDKRRGRDPEMGGKPRRKNPQEGLYNELQKDKMAEAYSEIGMKGERRRGKGHDGLYQGLSTATKDTYDALHMQALPPRLGSGEGRGSLLTCGDVEENPGPMVLGTIDLCSCFSAGLPKTEANWVNVISDLKKIEDLIQSMHIDATLYTESDVHPSCKVTAMKCFLLELQVISLESGDASIHDTVENLIILANNSLSSNGNVTESGCKECEELEEKNIKEFLQSFVHIVQMFINTSSGGGSGGGGSGGGGSGGGGSGGGSLQITCPPPMSVEHADIWVKSYSLYSRERYICNSGFKRKAGTSSLTECVLNKATNVAHWTTPSLKCIRDPALVHQRPAPPSTVTTAGVTPQPESLSPSGKEPAASSPSSNNTAATTAAIVPGSQLMPSKSPSTGTTEISSHESSHGTPSQTTAKNWELTASASHQPPGVYPQGHSDTTVAISTSTVLLCGLSAVSLLACYLKSRQTPPLASVEMEAMEALPVTWGTSSRDEDLENCSHHL

SEQ ID NO: 18 - protein, 971 aa, synthetic construct
  REGION 1..971: note = CAR Cd19/IL27
MYRMQLLSCIALSLALVTNSDIQLTQSPASLAVSLGQRATISCKASQSVDYDGDSYLNWYQQIPGQPPKLLIYDASNLVSGIPPRFSGSGSGTDFTLNIHPVEKVDAATYHCQQSTEDPWTFGGGTKLEIKGGGGSGGGGSGGGGSQVQLQQSGAELVRPGSSVKISCKASGYAFSSYWMNWVKQRPGQGLEWIGQIWPGDGDTNYNGKFKGKATLTADESSSTAYMQLSSLASEDSAVYFCARRETTTVGRYYYAMDYWGQGTTVTVSSSTTTPAPRPPTPAPTIASQPLSLRPEACRPAAGGAVHTRGLDFACDIYIWAPLAGTCGVLLLSLVITLYCKRGRKKLLYIFKQPFMRPVQTTQEEDGCSCRFPEEEEGGCELRVKFSRSADAPAYKQGQNQLYNELNLGRREEYDVLDKRRGRDPEMGGKPRRKNPQEGLYNELQKDKMAEAYSEIGMKGERRRGKGHDGLYQGLSTATKDTYDALHMQALPPRLGSGEGRGSLLTCGDVEENPGPMTPQLLLALVLWASCPPCSGRKGPPAALTLPRVQCRASRYPIAVDCSWTLPPAPNSTSPVSFIATYRLGMAARGHSWPCLQQTPTSTSCTITDVQLFSMAPYVLNVTAVHPWGSSSSFVPFITEHIIKPDPPEGVRLSPLAERQLQVQWEPPGSWPFPEIFSLKYWIRYKRQGAARFHRVGPIEATSFILRAVRPRARYYIQVAAQDLTDYGELSDWSLPATATMSLGKVPGVGVPGVGFPRPPGRPQLSLQELRREFTVSLHLARKLLAEVRGQAHRFAESHLPGVNLYLLPLGEQLPDVSLTFQAWRRLSDPERLCFISTTLQPFHALLGGLGTQGRWTNMERMQLWAMRLDLRDLQRHLRFQVLAAGFNLPEEEEEEEEEEEEERKGLLPGALGSALQGPAQVSWPQLLSTYRLLHSLELVLSRAVRELLLLSKAGHSVWPLGFPTLSPQPN

SEQ ID NO: 19 - DNA, 30 bp, synthetic construct
  misc_feature 1..30: note = ligante de elastina nucleotdeos da IL-17
  source 1..30: mol_type = other DNA
gttcctggagtaggggtacctggagtgggc

SEQ ID NO: 20 - DNA, 71 bp, synthetic construct
  misc_feature 1..71: note = ligante de elastina nucleotdeos da IL-15
  source 1..71: mol_type = other DNA
gcggcggcggcagcggcggcggcggcagcggcggcggcggcagcggcggcggcggcagcggcggcggcagc